European Patent Application EP 4 722 337 A1, published April 8, 2026. Title: Protocatechuic acid-producing Hydrogenophilus bacterium transformant. Applicant: 株式会社ＣＯ２資源化研究所. The sequence listing filed with the application follows.

SEQUENCE LISTING (40 sequences)

SEQ ID NO: 1 - DNA, 579 bp, Shewanella algae
  source 1..579: mol_type = genomic DNA
atgtccgtgacctccctatcgttcccctacggtgaaagtatccagtggttctcccccgaacaaagtcagcaactaccggcagcaccccttcacgactggctcctcgcaaccggctcccttaccaaacgtcttaaatcctgctgcaaccacttcgaagttaagctccttggcgaagcgatgctcccgagttccacacgtgaatggcagggtaaagaacacaaggcgatctggatccgtgaagttcttctttgcctcgatggtacaccgtgggttttcggccgcaccctcatcccggcaaaactcctcgaacaacagcagcgtctcggcaaacttggcacccgcccgctcggagaacttcttttcggcgacatcggcttcgaaccgggcgcgattgaagttgcgtccttcgattcgcaatcccgtatcgcgtcccttgcggatagtctcagtcaaccgaccacagaagcaatttggggccgtcgtcggtacttccacttccacgaacaacagctcatcgttggtgaaatcttcctcccggcagcagttgcggcgatcaaccaaggacccctaaccccgtga

SEQ ID NO: 2 - protein, 192 aa, Shewanella algae
MSVTSLSFPYGESIQWFSPEQSQQLPAAPLHDWLLATGSLTKRLKSCCNHFEVKLLGEAMLPSSTREWQGKEHKAIWIREVLLCLDGTPWVFGRTLIPAKLLEQQQRLGKLGTRPLGELLFGDIGFEPGAIEVASFDSQSRIASLADSLSQPTTEAIWGRRRYFHFHEQQLIVGEIFLPAAVAAINQGPLTP

SEQ ID NO: 3 - DNA, 1188 bp, Corynebacterium glutamicum
  source 1..1188: mol_type = genomic DNA
atgaaccacgtaccagtggcaattattggcgcaggaccagcaggactaaccctcgcccacctcctccaccttcaaggtgtggaatcaatcgtctttgaatcccgcacccgcaaggacgtcgaagaaaccgtccgagcaggcatcctggaacaaggcaccctgaatctgatgcgcgaaaccggagtcggcgcacgcatggaagcagaagccgatcacgatgaagcaatcgacatctccatcaacaatgagcgcacccgcattccgctgaccgaactcaccggccacaaggttgcgatctacccgcagcacgaatacctcaaagatttcattgccaagcgcatcgaagatggcggcgaactccttttcaccaccactgttgattccgtagaaaactacgaaggcgacctcgccaaggtgacctacaccgaagccgatggttcctccaccaccatcaccgccgactacgtcatcgcagctgacggctccaactccccttaccgcaagctgatcaccgaagacggtggcgtgcgcgcccgccatgaatacccttacgcatggttcggcattttggtggaagcaccaaaaacccaaaaggaactcatctacgcaacccaccctgagggctttgcgctgatctccacccgtaccgatgaaatccagcgctactacctgcagtgcaaccctgacgacaccccagacatgtggcccgatgaccgcatttgggaacagctgcacctgcgtgcggactcccctggcatcaccgtgtctgaagggcgcatctttgacaaggccgtgctgcgtttccgctccgcggtcaccgaaccaatgcaaaagggacgcctcttccttgctggcgatgctgcacacaccgtgccgccaaccggagctaagggcctcaacttggctgttgccgatgtctcagtactcgcgccagcactggttcgtgccctgaagaagaaggacaccggcttgctcgatagctacacctccctggcagtcccccgcatctggaaagcacagcacttctcctactggatgagctccatgctccacgcagtacccggcgaagatcactttgccacccagcgccgattcgctgaattgcgctccgtcctagaatcccaatccggccaacgctacctcgcagagcagtacgttgggcgcgacctaccacgcttcgaggtatga

SEQ ID NO: 4 - protein, 395 aa, Corynebacterium glutamicum
MNHVPVAIIGAGPAGLTLAHLLHLQGVESIVFESRTRKDVEETVRAGILEQGTLNLMRETGVGARMEAEADHDEAIDISINNERTRIPLTELTGHKVAIYPQHEYLKDFIAKRIEDGGELLFTTTVDSVENYEGDLAKVTYTEADGSSTTITADYVIAADGSNSPYRKLITEDGGVRARHEYPYAWFGILVEAPKTQKELIYATHPEGFALISTRTDEIQRYYLQCNPDDTPDMWPDDRIWEQLHLRADSPGITVSEGRIFDKAVLRFRSAVTEPMQKGRLFLAGDAAHTVPPTGAKGLNLAVADVSVLAPALVRALKKKDTGLLDSYTSLAVPRIWKAQHFSYWMSSMLHAVPGEDHFATQRRFAELRSVLESQSGQRYLAEQYVGRDLPRFEV

SEQ ID NO: 5 - DNA, 35 bp, synthetic construct
  source 1..35: mol_type = other DNA
ttttataacccgggccatcgactgcacggtgcacc

SEQ ID NO: 6 - DNA, 35 bp, synthetic construct
  source 1..35: mol_type = other DNA
tgctagcactgtttcctgtgtgaaattgttatccg

SEQ ID NO: 7 - DNA, 38 bp, synthetic construct
  source 1..38: mol_type = other DNA
ggaaacagtgctagcagatctggaggagaaaggcatat

SEQ ID NO: 8 - DNA, 72 bp, synthetic construct
  source 1..72: mol_type = other DNA
cagtgcggccgcaagcttgtcgacggagctcgaattcggatccgatatcagcatatgcgtttctcctccaga

SEQ ID NO: 9 - DNA, 80 bp, synthetic construct
  source 1..80: mol_type = other DNA
acaagcttgcggccgcactgcagcaccatcaccaccatcattgataagatccggctgctaacaaagcccgaaaggaagct

SEQ ID NO: 10 - DNA, 63 bp, synthetic construct
  source 1..63: mol_type = other DNA
tatttgaatcgagttattgctcagcggtggcagcagccaactcagcttcctttcgggctttgt

SEQ ID NO: 11 - DNA, 35 bp, synthetic construct
  source 1..35: mol_type = other DNA
taactcgattcaaataaaacgaaaggctcagtcga

SEQ ID NO: 12 - DNA, 35 bp, synthetic construct
  source 1..35: mol_type = other DNA
cctagatccgcggagtttgtagaaacgcaaaaagg

SEQ ID NO: 13 - DNA, 35 bp, synthetic construct
  source 1..35: mol_type = other DNA
acaaactccgcggatctaggtgaagatcctttttg

SEQ ID NO: 14 - DNA, 35 bp, synthetic construct
  source 1..35: mol_type = other DNA
cgtccgcggccagcaaaaggccaggaaccgtaaaa

SEQ ID NO: 15 - DNA, 35 bp, synthetic construct
  source 1..35: mol_type = other DNA
ttgctggccgcggacgtagaaagcctgtccgcaga

SEQ ID NO: 16 - DNA, 35 bp, synthetic construct
  source 1..35: mol_type = other DNA
ggcccgggttataaaagccagtcattaggcctatc

SEQ ID NO: 17 - DNA, 35 bp, synthetic construct
  source 1..35: mol_type = other DNA
aattgtcagataggcctaatgactggcttttataa

SEQ ID NO: 18 - DNA, 35 bp, synthetic construct
  source 1..35: mol_type = other DNA
tgacgccagaagcattggtgcaccgtgcagtcgat

SEQ ID NO: 19 - DNA, 19 bp, synthetic construct
  source 1..19: mol_type = other DNA
gatctggaggagaaacgca

SEQ ID NO: 20 - DNA, 17 bp, synthetic construct
  source 1..17: mol_type = other DNA
tatgcgtttctcctcca

SEQ ID NO: 21 - DNA, 35 bp, synthetic construct
  source 1..35: mol_type = other DNA
gaggccatctaggccatgagtaagtctgacggaac

SEQ ID NO: 22 - DNA, 35 bp, synthetic construct
  source 1..35: mol_type = other DNA
atccggcacccatatctgaaccggacgcaaacccg

SEQ ID NO: 23 - DNA, 35 bp, synthetic construct
  source 1..35: mol_type = other DNA
ttcagatatgggtgccggatacccgccgcccgggc

SEQ ID NO: 24 - DNA, 35 bp, synthetic construct
  source 1..35: mol_type = other DNA
aaggccttcatggccttatttcgcgattcccaaga

SEQ ID NO: 25 - DNA, 44 bp, synthetic construct
  source 1..44: mol_type = other DNA
gcagatctggaggagaaacgcatatgagtgtgaccagtttaagc

SEQ ID NO: 26 - DNA, 43 bp, synthetic construct
  source 1..43: mol_type = other DNA
cttgtcgacggagctcgaattctcaaggcgtaagttggccttg

SEQ ID NO: 27 - DNA, 20 bp, synthetic construct
  source 1..20: mol_type = other DNA
gaattcgagctccgtcgaca

SEQ ID NO: 28 - DNA, 20 bp, synthetic construct
  source 1..20: mol_type = other DNA
atgcgtttctcctccagatc

SEQ ID NO: 29 - DNA, 1200 bp, Meiothermus timidus
  source 1..1200: mol_type = genomic DNA
atggctagggtgggcgtggtgggggcggggccggcggggttgttgctggcctacctgctgcaccgcgagggccttgaggtggtggtcttcgaggccaaaagccgcgagtacctggagacaagcccccaccgcatccgcgcgggggtgctggagtggggcagccaggagattctgcgccgggccgggctgggacagcggatgctcgagcagggcttagagcaccggggggtctacctggctttcgacagggccctgcaccggctggactttcccagcctcaccggcaagagcatctgggtctacagccagcagttcgtggtgcaggacatgataaggctccacctggcccagggcggggcgattcgctttgagcacgaggtgctgggcctggaggaggacgcggggggtctttgggtggtctaccgtacccccgagggcgcgaccgagcggatgcgctgcgatttcgtggtgggggccgacggctcgcacagccggctgcgggcccagataccggaggcccggctgcaccagaagaactaccccttcgcctggctgggcatcctggccgaggccccgcccgccgccgaggagctcatctacgccagccacccccgcggctttgccctcttcagcatgcgctcgcccacccgctcgaggaactacctgcaagtgggggtggaggagcggctcgaggactggcccgaggagcgcatctgggccgagctgaacgagcggcttgggggggtggccgaggtgcgcccggggcccctgttggaaaaaagcctcacccccctgcgctccttggtgctggagcccatgcagcacggccgcttcttcctgatgggcgacgcggcccacgtggtgccgcccaccggggccaagggcatgaacctggccctctctgatgcggtgcttttgtaccgggcgctactggcctactaccgccggggcgaggagggccatctgttgcgctacacccaggacgcgctgcgccacgtctggcaggccgagctcttctcctacttcatgaccaccctgctccacacccccaccgaccccttcgacgacgggctgcgcaccgcccagctccgccacctggccgaaagcccccacctccagcgcttcctggccgagaactacgtgggcctctacaccagcggacgctaccccgggtgggtgggggagggggtctcggcctag

SEQ ID NO: 30 - DNA, 1197 bp, Amycolatopsis thermoflava
  source 1..1197: mol_type = genomic DNA
atgacgcgcacacaggtcgggatcatcggcgccgggccggccggtctgctcttgtcgtacctgctgcacgccgagggtgtcgacgccgtggtcctcgagacgcgcagccgcgcctacgtggagaagcgggtgcgcgccggggtctgcgagcacccgacggtcgagctgctgcgggagatcggcgtcggcacgaggttggatgccgaaggcctgccgcaccacgggttttcgctgcggttcgacgggcaggaccaccgcatcgcgctcaccgagctgaccggcaagtcgatcacggtgtacgggcagcaggagatcgtcaaggacctgatcgccgcgcacgaggccaagggctacccgatccggttcgaggtcagcgacgtcgaactgcacgacgtggacaccgacaacccgcgcatcacctaccgggactccgacggcgcggcgcagaccctggcgtgcgacgtgatcgccgggtgcgacggcttccacggcgtcagccggccgacgatccccgcagacaaggtcaagaccttcgaccgcgagtatccgttcgcctggctgggcgtgctggcgcagaccccgccgtcgcacgaggagctgatctacacccaccacgagcgcgggttcgccctgcacagcatgcgctcgccggagatcacgcggctctacctgcaggtgcccagcgacgagaagatcgaaaactggtccgacgaccgcatctggtccgagctggacgtccggctcaccacgaacgcgcacgacttcgtgctgcgcgaggggccgatcctggacaagggcatcacgccgatgcgcagcttcgtcaccgaacccatgcagtacggacgactgttcctcgccggcgacgcggcgcacatcgtgccgccgaccggggcgaagggcatgaacctggccgtcgccgacgtacgcgtgctgtcccgtgcgctggtggaactgttgcagcacaagcggagcgagctggcggagtcctattcggacacctgcctgcggcgcgtgtggcgggccgagcacttctcctggtacatgacctcgatgctgcacgtggacccgtcggcggacgacttcacccggcggctccagctgtcgcaactgcggtacacggcgtcgtcccgcgccgcggcgacgagcgtggcggagaactacgtggggctgccgttcgcctggacgagtaatgcgtaa

SEQ ID NO: 31 - DNA, 42 bp, synthetic construct
  source 1..42: mol_type = other DNA
cagatctggaggagaaacgcatatgaaccacgtaccagtggc

SEQ ID NO: 32 - DNA, 43 bp, synthetic construct
  source 1..43: mol_type = other DNA
cttgtcgacggagctcgaattcttatacctcgaagcgtggtag

SEQ ID NO: 33 - DNA, 43 bp, synthetic construct
  source 1..43: mol_type = other DNA
cagatctggaggagaaacgcatatggctagggtgggcgtggtg

SEQ ID NO: 34 - DNA, 42 bp, synthetic construct
  source 1..42: mol_type = other DNA
gtcgacggagctcgaattcctaggccgagaccccctccccca

SEQ ID NO: 35 - DNA, 44 bp, synthetic construct
  source 1..44: mol_type = other DNA
gatctggaggagaaacgcatatgacgcgcacacaggtcgggatc

SEQ ID NO: 36 - DNA, 44 bp, synthetic construct
  source 1..44: mol_type = other DNA
cttgtcgacggagctcgaattcttacgcattactcgtccaggcg

SEQ ID NO: 37 - DNA, 21 bp, synthetic construct
  source 1..21: mol_type = other DNA
ccgcggatctaggtgaagatc

SEQ ID NO: 38 - DNA, 27 bp, synthetic construct
  source 1..27: mol_type = other DNA
agtttgtagaaacgcaaaaaggccatc

SEQ ID NO: 39 - DNA, 44 bp, synthetic construct
  source 1..44: mol_type = other DNA
gcctttttgcgtttctacaaactcccatcgactgcacggtgcac

SEQ ID NO: 40 - DNA, 40 bp, synthetic construct
  source 1..40: mol_type = other DNA
gtcatgagattatcaaaaaggatcttcacctagatccgcg